European Patent Specification EP 3 230 435 B1, published November 29, 2023. Title: Method for removing DNA from fermentation products. Applicant: BASF SE. The sequence listing filed with the application follows.

SEQUENCE LISTING (29 sequences)

SEQ ID NO: 1 - DNA, 708 bp, Eremothecium gossypii
atgtttaccggtatagtggaacacattggcactgttgctgagtacttggagaacgatgccagcgaggcaggcggcaacggtgtgtcagtccttatcaaggatgcggctccgatactggcggattgccacatcggtgactcgattgcatgcaatggtatctgcctgacggtgacggagttcacggccgatagcttcaaggtcgggatcgcaccagaaacagtttatcggacggaagtcagcagctggaaagctggctccaagatcaacctagaaagggccatctcggacgacaggcgctacggcgggcactacgtgcagggccacgtcgactcggtggcctctattgtatccagagagcacgacgggaactctatcaactttaagtttaaactgcgcgatcaagagtacgagaagtacgtagtagaaaagggttttgtggcgatcgacggtgtgtcgctgactgtaagcaagatggatccagatggctgtttctacatctcgatgattgcacacacgcagaccgctgtagcccttccactgaagccggacggtgccctcgtgaacatagaaacggatgttaacggcaagctagtagagaagcaggttgcacagtacctgaatgcgcagctggaaggtgagagctcgccattgcagcgcgtgctcgaaaggattattgaatccaagcttgctagcatctcaaataagtga

SEQ ID NO: 2 - DNA, 22 bp, artificial
  primer P1
atgtttaccggtatagtggaac

SEQ ID NO: 3 - DNA, 25 bp, artificial
  primer P2
tcacttatttgagatgctagcaagc

SEQ ID NO: 4 - DNA, 1758 bp, Eremothecium gossypii
atggaaaacacatcgcaggatgagagtcgcaaaagacaggtcgcttcgaacttgagcagcgatgccgatgagggctcgccggcagttacgaggccggttaaaatcaccaaacgcctcaggaagaagaacctcgggacaggcgagctacgggacaaagcaggattcaagttgaaggtgcaagacgtgagcaaaaaccgtcacagacaggtcgatccggaatacgaagtcgtggtagatggcccgatgcgcaagatcaaaccgtatttcttcacatacaagactttctgcaaggagcgctggagagatcggaagttgcttgatgtgtttgtggatgaatttcgggaccgcgataggccttactacgagaaagtcatcggttcgggtggtgtgctcctgaacggtaagtcatcgacgttagatagcgtattgcgtaatggagacctcatttcgcacgagctgcaccgtcatgagccaccggtctcctctaggccgattaggacggtgtacgaagatgatgacatcctggtgattgacaagcccagcgggattccagcccatcccaccgggcgttaccgcttcaactccattacgaaaatacttgaaaaacagcttggatacactgttcatccatgtaaccgactggaccgcctaaccagtggcctaatgttcttggcaaaaactccaaagggagccgatgagatgggtgatcagatgaaggcgcgcgaagtgaagaaagaatatgttgcccgggttgttggggaatttcctataggtgagatagttgtggatatgccactgaagactatagagccgaagcttgccctaaacatggtttgcgacccggaagacgaagcgggcaagggcgctaagacgcagctcaaaagaatcagctacgatggacaaacgagcatagtcaagtgccaaccgtacacgggccggacgcatcagatccgtgttcacttgcaatacctgggcttcccaattgccaacgatccgatttattccaatccgcacatatggggcccaagtctgggcaaggaatgcaaagcagactacaaggaggtcatccaaaaactaaacgaaattggtaagactaaatctgcggaaagttggtaccattctgattcccaaggtgaagttttgaaaggggaacaatgcgatgaatgtggcaccgaactgtacactgacccgggcccgaatgatcttgacttatggttgcatgcatatcggtatgaatccactgaactggatgagaacggtgctaaaaagtggagttactctactgcgtttcctgagtgggctcttgagcagcacggcgacttcatgcggcttgccatcgaacaggctaagaaatgcccacccgcgaagacatcatttagcgttggtgccgtgttagttaatgggaccgagattttggccactggttactcacgggagctggaaggcaacacgcacgctgaacaatgtgcacttcaaaaatattttgaacaacataaaaccgacaaggttcctattggtacagtaatatacacgactatggagccttgttctctccgtctcagtggtaataaaccgtgtgttgagcgtataatctgccagcagggtaatattactgctgtttttgttggcgtacttgagccagacaacttcgtgaagaacaatacaagtcgtgcgctattggaacaacatggtatagactatattcttgtccctgggtttcaagaagaatgtactgaagccgcattgaagggtcattga

SEQ ID NO: 5 - DNA, 26 bp, artificial
  primer P3
atggaaaacacatcgcaggatgagag

SEQ ID NO: 6 - DNA, 24 bp, artificial
  primer P4
tcaatgacccttcaatgcggcttc

SEQ ID NO: 7 - DNA, 519 bp, Eremothecium gossypii
atgattaagggattaggcgaagttgatcaaacctacgatgcgagctctgtcaaggttggcattgtccacgcgagatggaacaagactgtcattgacgctctcgtccaaggtgcaattgagaaactgcttgctatgggagtgaaggagaagaatatcactgtaagcaccgttccaggtgcgtttgaactaccatttggcactcagcggtttgccgagctgaccaaggcaagtggcaagcatttggacgtggtcatcccaattggagtcctgatcaaaggcgactcaatgcactttgaatatatatcagactctgtgactcatgccttaatgaacctacagaagaagattcgtcttcctgtcatttttggtttgctaacgtgtctaacagaggaacaagcgttgacacgtgcaggcctcggtgaatctgaaggcaagcacaaccacggtgaagactggggtgctgctgccgtggagatggctgtaaagtttggcccacgcgccgaacaaatgaagaagtga

SEQ ID NO: 8 - DNA, 22 bp, artificial
  primer P5
atgattaagggattaggcgaag

SEQ ID NO: 9 - DNA, 20 bp, artificial
  primer P6
tcacttcttcatttgttcgg

SEQ ID NO: 10 - DNA, 639 bp, Eremothecium gossypii
atgacaagcccatgcactgatatcggtaccgctatagagcagttcaagcaaaataagatgatcatcgtcatggaccacatctcgagagaaaacgaggccgatctaatatgtgcagcagcgcacatgactgccgagcaaatggcatttatgattcggtattcctcgggctacgtttgcgctccaatgaccaatgcgattgccgataagctagacctaccgctcatgaacacattgaaatgcaaggctttctccgatgacagacacagcactgcgtatacaatcacctgtgactatgcgcacgggacgacgacaggtatctccgcacgtgaccgggcgttgacctgtaatcagttggcgaacccggagtccaaggctaccgacttcacgaagccaggccacattgtgccattgcgtgcccgtgacggcggcgtgctcgagcgtgacgggcacaccgaagcggcgctcgacttgtgcagactagcgggtgtgccagaggtcgctgctatttgtgaattagtaagcgaaagggacgtcgggctgatgatgactttggatgagtgtatagaattcagcaagaagcacggtcttgccctcatcaccgtcgatgacctgaaggctgcagttgccgccaagcagtag

SEQ ID NO: 11 - DNA, 1083 bp, Eremothecium gossypii
atgtgcaaggccggtttcgccggtgacgacgctccccgggctgtgttcccttcgatcgtcggcagacccagacaccagggtatcatggtgggtatgggccagaaggactcctatgtgggcgatgaggcgcaatcgaagagaggtatcttgacgttgcgttacccaatcgagcacggtatcgtcacaaactgggatgacatggagaagatctggcaccacaccttttacaacgaattgagagtggccccagaggaacacccagtgttgttgacggaggcgcctatgaaccctaagtcgaacagagaaaagatgacgcagatcatgtttgaaactttcaacgtgcctgccttctacgtgtccattcaggccgtcttgtcgctatactcttctggtagaacgacgggtattgtgttggactccggtgacggtgttacccacgttgttcctatctacgctggtttctcgttgccacacgccattttgagaattgacttggccggcagagatatgaccgactacttgatgaagattctatcggaacgtggctactccttttccaccactgcagagagagaaattgtccgtgacatcaaagagaagctatgttacgtcgccttggacttcgaacaagagatgcagactgctgcccagtcttcggccatcgagaagtcctacgagctacctgacggtcaggtgatcactatcggtaacgaaagattcagagctccagaagctttgttccatccatctgtgttgggcttggaggctgccggtattgatcaaaccacctacaactccatcatgaagtgtgacgtggacgtcagaaaggagctctacggtaacattgtgatgtctggtggtactactatgttccctggtatcgccgagagaatgcagaaggagatcacggccttggcgccatcctccatgaaggtgaagattatcgctccaccagagagaaagtactccgtctggatcggtggttctatcttggcctctctaaccaccttccagcagatgtggatctcgaagcaggaatacgatgagtctgggccatccatcgttcaccacaagtgtttctaa

SEQ ID NO: 12 - DNA, 19 bp, artificial
  primer P9
gatgacagacacagcactg

SEQ ID NO: 13 - DNA, 20 bp, artificial
  primer P10
ctactgcttggcggcaactg

SEQ ID NO: 14 - DNA, 20 bp, artificial
  primer P11
gatgacgcagatcatgtttg

SEQ ID NO: 15 - DNA, 18 bp, artificial
  primer P12
ccagaagagtatagcgac

SEQ ID NO: 16 - DNA, 21 bp, artificial
  primer P13
tgtgaattagtaagcgaaagg

SEQ ID NO: 17 - DNA, 18 bp, artificial
  primer P14
gcagccttcaggtcatcg

SEQ ID NO: 18 - DNA, 17 bp, artificial
  primer P15
gcagcagcgcacatgac

SEQ ID NO: 19 - DNA, 20 bp, artificial
  primer P16
tgcggagatacctgtcgtcg

SEQ ID NO: 20 - DNA, 21 bp, artificial
  primer P17
gatgaagattctatcggaacg

SEQ ID NO: 21 - DNA, 20 bp, artificial
  primer P18
gcatctcttgttcgaagtcc

SEQ ID NO: 22 - DNA, 1980 bp, Bacillus subtilis
atgtttgcaaaacgattcaaaacctctttactgccgttattcgctggatttttattgctgtttcatttggttctggcaggaccggcggctgcgagtgctgaaacggcgaacaaatcgaatgagcttacagcaccgtcgatcaaaagcggaaccattcttcatgcatggaattggtcgttcaatacgttaaaacacaatatgaaggatattcatgatgcaggatatacagccattcagacatctccgattaaccaagtaaaggaagggaatcaaggagataaaagcatgtcgaactggtactggctgtatcagccgacatcgtatcaaattggcaaccgttacttaggtactgaacaagaatttaaagaaatgtgtgcagccgctgaagaatatggcataaaggtcattgttgacgcggtcatcaatcataccaccagtgattatgccgcgatttccaatgaggttaagagtattccaaactggacacatggaaacacacaaattaaaaactggtctgatcgatgggatgtcacgcagaattcattgctcgggctgtatgactggaatacacaaaatacacaagtacagtcctatctgaaacggttcttagacagggcattgaatgacggggcagacggttttcgatttgatgccgccaaacatatagagcttccagatgatggcagttacggcagtcaattttggccgaatatcacaaatacatctgcagagttccaatacggagaaatcctgcaggatagtgcctccagagatgctgcatatgcgaattatatggatgtgacagcgtctaactatgggcattccataaggtccgctttaaagaatcgtaatctgggcgtgtcgaatatctcccactatgcatctgatgtgtctgcggacaagctagtgacatgggtagagtcgcatgatacgtatgccaatgatgatgaagagtcgacatggatgagcgatgatgatatccgtttaggctgggcggtgatagcttctcgttcaggcagtacgcctcttttcttttccagacctgagggaggcggaaatggtgtgaggttcccggggaaaagccaaataggcgatcgcgggagtgctttatttgaagatcaggctatcactgcggtcaatagatttcacaatgtgatggctggacagcctgaggaactctcgaacccgaatggaaacaaccagatatttatgaatcagcgcggctcacatggcgttgtgctggcaaatgcaggttcatcctctgtctctatcaatacggcaacaaaattgcctgatggcaggtatgacaataaagctggagcgggttcatttcaagtgaacgatggtaaactgacaggcacgatcaatgccaggtctgtagctgtgctttatcctgatgatattgcaaaagcgcctcatgttttccttgagaattacaaaacaggtgtaacacattctttcaatgatcaactgacgattaccttgcgtgcagatgcgaatacaacaaaagccgtttatcaaatcaataatggaccagagacggcgtttaaggatggagatcaattcacaatcggaaaaggagatccatttggcaaaacatacaccatcatgttaaaaggaacgaacagtgatggtgtaacgaggaccgagaaatacagttttgttaaaagagatccagcgtcggccaaaaccatcggctatcaaaatccgaatcattggagccaggtaaatgcttatatctataaacatgatgggagccgagtaattgaattgaccggatcttggcctggaaaaccaatgactaaaaatgcagacggaatttacacgctgacgctgcctgcggacacggatacaaccaacgcaaaagtgatttttaataatggcagcgcccaagtgcccggtcagaatcagcctggctttgattacgtgctaaatggtttatataatgactcgggcttaagcggttctcttccccattga

SEQ ID NO: 23 - DNA, 17 bp, artificial
  primer P19
gtgctggcaaatgcagg

SEQ ID NO: 24 - DNA, 22 bp, artificial
  primer P20
gctacagacctggcattgatcg

SEQ ID NO: 25 - DNA, 20 bp, artificial
  primer P21
tgccgttattcgctggattt

SEQ ID NO: 26 - DNA, 20 bp, artificial
  primer P22
atcgcggcataatcactggt

SEQ ID NO: 27 - DNA, 1266 bp, Corynebacterium glutamicum
gtggccctggtcgtacagaaatatggcggttcctcgcttgagagtgcggaacgcattagaaacgtcgctgaacggatcgttgccaccaagaaggctggaaatgatgtcgtggttgtctgctccgcaatgggagacaccacggatgaacttctagaacttgcagcggcagtgaatcccgttccgccagctcgtgaaatggatatgctcctgactgctggtgagcgtatttctaacgctctcgtcgccatggctattgagtcccttggcgcagaagcccaatctttcacgggctctcaggctggtgtgctcaccaccgagcgccacggaaacgcacgcattgttgatgtcactccaggtcgtgtgcgtgaagcactcgatgagggcaagatctgcattgttgctggtttccagggtgttaataaagaaacccgcgatgtcaccacgttgggtcgtggtggttctgacaccactgcagttgcgttggcagctgctttgaacgctgatgtgtgtgagatttactcggacgttgacggtgtgtataccgctgacccgcgcatcgttcctaatgcacagaagctggaaaagctcagcttcgaagaaatgctggaacttgctgctgttggctccaagattttggtgctgcgcagtgttgaatacgctcgtgcattcaatgtgccacttcgcgtacgctcgtcttatagtaatgatcccggcactttgattgccggctctatggaggatattcctgtggaagaagcagtccttaccggtgtcgcaaccgacaagtccgaagccaaagtaaccgttctgggtatttccgataagccaggcgaggctgcgaaggttttccgtgcgttggctgatgcagaaatcaacattgacatggttctgcagaacgtctcttctgtagaagacggcaccaccgacatcaccttcacctgccctcgttccgacggccgccgcgcgatggagatcttgaagaagcttcaggttcagggcaactggaccaatgtgctttacgacgaccaggtcggcaaagtctccctcgtgggtgctggcatgaagtctcacccaggtgttaccgcagagttcatggaagctctgcgcgatgtcaacgtgaacatcgaattgatttccacctctgagattcgtatttccgtgctgatccgtgaagatgatctggatgctgctgcacgtgcattgcatgagcagttccagctgggcggcgaagacgaagccgtcgtttatgcaggcaccggacgctaa

SEQ ID NO: 28 - DNA, 20 bp, artificial
  primer P23
ggagatcttgaagaagcttc

SEQ ID NO: 29 - DNA, 20 bp, artificial
  primer P24
gatcatcttcacggatcagc